European Patent Application EP 4 324 902 A2, published February 21, 2024. Title: Fast methods for preparing cereal extracts. Applicant: Carlsberg A/S. Application EP. The sequence listing filed with the application follows.

SEQUENCE LISTING (24 sequences)

SEQ ID NO: 1 - protein, 947 aa, Hordeum vulgare
MAPAVAGGGRVRSNEPVAAAAAAPAASGKPCVCGFQVCACTGSAAVASAASSLDMDIVAMGQIGAVNDESWVGVELGEDGETDESGAAVDDRPVFRTEKIKGVLLHPYRVLIFVRLIAFTLFVIWRISHKNPDAMWLWVTSICGEFWFGFSWLLDQLPKLNPINRVPDLAVLRQRFDRPDGTSTLPGLDIFVTTADPIKEPILSTANSVLSILAADYPVDRNTCYVSDDSGMLLTYEALAESSKFATLWVPFCRKHGIEPRGPESYFELKSHPYMGRAQDEFVNDRRRVRKEYDEFKARINSLEHDIKQRNDGYNAAIAHSQGVPRPTWMADGTQWEGTWVDASENHRRGDHAGIVLVLLNHPSHRRQTGPPASADNPLDLSGVDVRLPMLVYVSREKRPGHDHQKKAGAMNALTRASALLSNSPFILNLDCDHYINNSQALRAGICFMVGRDSDTVAFVQFPQRFEGVDPTDLYANHNRIFFDGTLRALDGMQGPIYVGTGCLFRRITVYGFDPPRINVGGPCFPRLAGLFAKTKYEKPGLEMTTAKAKAAPVPAKGKHGFLPLPKKTYGKSDAFVDTIPRASHPSPYAAAAEGIVADEATIVEAVNVTAAAFEKKTGWGKEIGWVYDTVTEDVVTGYRMHIKGWRSRYCSIYPHAFIGTAPINLTERLFQVLRWSTGSLEIFFSKNNPLFGSTYLHPLQRVAYINITTYPFTAIFLIFYTTVPALSFVTGHFIVQRPTTMFYVYLGIVLSTLLVIAVLEVKWAGVTVFEWFRNGQFWMTASCSAYLAAVCQVLTKVIFRRDISFKLTSKLPSGDEKKDPYADLYVVRWTPLMITPIIIIFVNIIGSAVAFAKVLDGEWTHWLKVAGGVFFNFWVLFHLYPFAKGILGKHGKTPVVVLVWWAFTFVITAVLYINIPHMHTSGGKHTTVHGHHGKKLVDTGLYGWLH

SEQ ID NO: 2 - DNA, 2844 bp, Hordeum vulgare
  source 1..2844: mol_type = genomic DNA
atggcgccagcggtggccggagggggccgcgtgcggagcaatgagccggttgctgctgctgccgccgcgccggcggccagcggcaagccctgcgtgtgcggcttccaggtttgcgcctgcacggggtcggccgcggtggcctccgccgcctcgtcgctggacatggacatcgtggccatggggcagatcggcgccgtcaacgacgagagctgggtgggcgtggagctcggcgaagatggcgagaccgacgaaagcggtgccgccgttgacgaccgccccgtattccgcaccgagaagatcaagggtgtcctcctccacccctaccgggtgctgattttcgttcgtctgatcgccttcacgctgttcgtgatctggcgtatctcccacaagaacccagacgcgatgtggctgtgggtgacatccatctgcggcgagttctggttcggtttctcgtggctgctagatcagctgcccaagctgaaccccatcaaccgcgtgccggacctggcggtgctgcggcagcgcttcgaccgccccgacggcacctccacgctcccggggctggacatcttcgtcaccacggccgaccccatcaaggagcccatcctctccaccgccaactcggtgctctccatcctggccgccgactaccccgtggaccgcaacacatgctacgtctccgacgacagtggcatgctgctcacctacgaggccctggcagagtcctccaagttcgccacgctctgggtgcccttctgccgcaagcacgggatcgagcccaggggtccggagagctacttcgagctcaagtcacacccttacatggggagagcccaggacgagttcgtcaacgaccgccgccgcgttcgcaaggagtacgacgagttcaaggccaggatcaacagcctggagcatgacatcaagcagcgcaacgacgggtacaacgccgccattgcccacagccaaggcgtgccccggcccacctggatggcggacggcacccagtgggagggcacatgggtcgacgcctccgagaaccaccgcaggggcgaccacgccggcatcgtactggtgctgctgaaccacccgagccaccgccggcagacgggcccgccggcgagcgctgacaacccactggacttgagcggcgtggatgtgcgtctccccatgctggtgtacgtgtcccgtgagaagcgccccgggcacgaccaccagaagaaggccggtgccatgaacgcgcttacccgcgcctcggcgctgctctccaactcccccttcatcctcaacctcgactgcgatcattacatcaacaactcccaggcccttcgcgccggcatctgcttcatggtgggacgggacagcgacacggttgccttcgtccagttcccgcagcgcttcgagggcgtcgaccccaccgacctctacgccaaccacaaccgcatcttcttcgacggcaccctccgtgccctggacggcatgcagggccccatctacgtcggcactgggtgtctcttccgccgcatcaccgtctacggcttcgacccgccgaggatcaacgtcggcggtccctgcttccccaggctcgccgggctcttcgccaagaccaagtacgagaagcccgggctcgagatgaccacggccaaggccaaggccgcgcccgtgcccgccaagggtaagcacggcttcttgccactgcccaagaagacgtacggcaagtcggacgccttcgtggacaccatcccgcgcgcgtcgcacccgtcgccctacgccgcggcggctgaggggatcgtggccgacgaggcgaccatcgtcgaggcggtgaacgtgacggccgccgcgttcgagaagaagaccggctggggcaaagagatcggctgggtgtacgacaccgtcacggaggacgtggtcaccggctaccggatgcatatcaaggggtggcggtcacgctactgctccatctacccacacgccttcatcggcaccgcccccatcaacctcacggagaggctcttccaggtgctccgctggtccacgggatccctcgagatcttcttctccaagaacaacccgctcttcggcagcacatacctccacccgctgcagcgcgtcgcctacatcaacatcaccacttaccccttcaccgccatcttcctcatcttctacaccaccgtgccggcgctatccttcgtcaccggccacttcatcgtgcagcgcccgaccaccatgttctacgtctacctgggcatcgtgctatccacgctgctcgtcatcgccgtgctggaggtcaagtgggccggggtcacagtcttcgagtggttcaggaacggccagttctggatgacagcaagttgctccgcctacctcgccgccgtctgccaggtgctgaccaaggtgatattccggcgggacatctccttcaagctcacatccaagctaccctcgggagacgagaagaaggacccctacgccgacctctacgtggtgcgctggacgccgctcatgattacacccatcatcatcatcttcgtcaacatcatcggatccgccgtggccttcgccaaggttctcgacggcgagtggacgcactggctcaaggtcgccggcggcgtcttcttcaacttctgggtgctcttccacctctaccccttcgccaagggcatcctggggaagcacggaaagacgccagtcgtggtgctcgtctggtgggcattcaccttcgtcatcaccgccgtgctctacatcaacatcccccacatgcatacctcgggaggcaagcacacaacggtgcatggtcaccatggcaagaagttggtcgacacagggctctatggctggctccattga

SEQ ID NO: 3 - DNA, 18 bp, synthetic construct
  misc_feature 1..18: note = AMY1 Fwd primer
  source 1..18: mol_type = other DNA
gggtcatgcagggatatg

SEQ ID NO: 4 - DNA, 19 bp, synthetic construct
  misc_feature 1..19: note = AMY1 Rev primer
  source 1..19: mol_type = other DNA
cccagtcgaagaaatgatc

SEQ ID NO: 5 - DNA, 19 bp, synthetic construct
  misc_feature 1..19: note = AMY1 Probe (FAM)
  source 1..19: mol_type = other DNA
tacatcctcacgcacccag

SEQ ID NO: 6 - DNA, 18 bp, synthetic construct
  misc_feature 1..18: note = BGL2 Fwd primer
  source 1..18: mol_type = other DNA
taccagaacctgttcgac

SEQ ID NO: 7 - DNA, 16 bp, synthetic construct
  misc_feature 1..16: note = BGL2 Rev primer
  source 1..16: mol_type = other DNA
acaccaccagcttcac

SEQ ID NO: 8 - DNA, 18 bp, synthetic construct
  misc_feature 1..18: note = BGL2 Probe (FAM)
  source 1..18: mol_type = other DNA
accgtggacgccttctac

SEQ ID NO: 9 - DNA, 15 bp, synthetic construct
  misc_feature 1..15: note = AGL97 Fwd primer
  source 1..15: mol_type = other DNA
gagtcgccggagatg

SEQ ID NO: 10 - DNA, 17 bp, synthetic construct
  misc_feature 1..17: note = AGL97 Rev primer
  source 1..17: mol_type = other DNA
gacttcaccttgatggc

SEQ ID NO: 11 - DNA, 20 bp, synthetic construct
  misc_feature 1..20: note = AGL97 Probe (FAM)
  source 1..20: mol_type = other DNA
catggtaaggttcagctgcg

SEQ ID NO: 12 - DNA, 18 bp, synthetic construct
  misc_feature 1..18: note = LD Fwd primer
  source 1..18: mol_type = other DNA
cttcgatggggtttgaac

SEQ ID NO: 13 - DNA, 18 bp, synthetic construct
  misc_feature 1..18: note = LD Rev primer
  source 1..18: mol_type = other DNA
ccgatttcctcaccaaag

SEQ ID NO: 14 - DNA, 21 bp, synthetic construct
  misc_feature 1..21: note = LD Probe (FAM)
  source 1..21: mol_type = other DNA
cctgtgcaggtgaattcatca

SEQ ID NO: 15 - DNA, 18 bp, synthetic construct
  misc_feature 1..18: note = RefA Fwd primer
  source 1..18: mol_type = other DNA
gtctattgcttcctctgc

SEQ ID NO: 16 - DNA, 18 bp, synthetic construct
  misc_feature 1..18: note = RefA Rev primer
  source 1..18: mol_type = other DNA
gatgaccgaagccttaac

SEQ ID NO: 17 - DNA, 17 bp, synthetic construct
  misc_feature 1..17: note = RefA Probe (HEX)
  source 1..17: mol_type = other DNA
tgcgggcggctatcaaa

SEQ ID NO: 18 - protein, 20 aa, synthetic construct
  REGION 1..20: note = Oligopeptide fragment
RVLIFVRLIAFTLFVIWRIS

SEQ ID NO: 19 - protein, 22 aa, synthetic construct
  REGION 1..22: note = Oligopeptide fragment
LWVTSICGEFWFGFSWLLDQLP

SEQ ID NO: 20 - protein, 12 aa, synthetic construct
  REGION 1..12: note = Oligopeptide fragment
LQRVAYINITTY

SEQ ID NO: 21 - protein, 17 aa, synthetic construct
  REGION 1..17: note = Oligopeptide fragment
  SITE 14: note = MISC_FEATURE - Xaa is U
AIFLIFYTTVPALXFVT

SEQ ID NO: 22 - protein, 18 aa, synthetic construct
  REGION 1..18: note = Oligopeptide fragment
TMFYVYLGIVLSTLLVIA

SEQ ID NO: 23 - protein, 23 aa, synthetic construct
  REGION 1..23: note = Oligopeptide sequence
ITPIIIIFVNIIGSAVAFAKVLD

SEQ ID NO: 24 - protein, 20 aa, synthetic construct
  REGION 1..20: note = Oligopeptide sequence
LKVAGGVFFNFWVLFHLYPF